European Patent Specification EP 3 787 661 B1, published October 18, 2023. Title: COMPOSITIONS AND METHODS FOR TREATING GLIOBLASTOMA. Applicant: TEL HASHOMER MEDICAL RESEARCH INFRASTRUCTURE AND SERVICES LTD. The sequence listing filed with the application follows.

SEQUENCE LISTING (17 sequences)

SEQ ID NO: 1 - protein, 4 aa, Artificial Sequence
  Peptide
LDPR

SEQ ID NO: 2 - protein, 5 aa, Artificial Sequence
  Peptide
TLDPR

SEQ ID NO: 3 - protein, 6 aa, Artificial Sequence
  Peptide
ATLDPR

SEQ ID NO: 4 - protein, 7 aa, Artificial Sequence
  Peptide
NATLDPR

SEQ ID NO: 5 - protein, 8 aa, Artificial Sequence
  Peptide
TNATLDPR

SEQ ID NO: 6 - protein, 9 aa, Artificial Sequence
  Peptide
ATNATLDPR

SEQ ID NO: 7 - protein, 10 aa, Artificial Sequence
  Peptide
KATNATLDPR

SEQ ID NO: 8 - protein, 11 aa, Artificial Sequence
  Peptide
SKATNATLDPR

SEQ ID NO: 9 - protein, 12 aa, Artificial Sequence
  Peptide
ESKATNATLDPR

SEQ ID NO: 10 - protein, 13 aa, Artificial Sequence
  Peptide
PESKATNATLDPR

SEQ ID NO: 11 - protein, 14 aa, Artificial Sequence
  Peptide
RPESKATNATLDPR

SEQ ID NO: 12 - protein, 15 aa, Artificial Sequence
  Peptide
RRPESKATNATLDPR

SEQ ID NO: 13 - protein, 16 aa, Artificial Sequence
  Peptide
ARRPESKATNATLDPR

SEQ ID NO: 14 - protein, 17 aa, Artificial Sequence
  Peptide
RARRPESKATNATLDPR

SEQ ID NO: 15 - protein, 18 aa, Artificial Sequence
  Peptide
TRARRPESKATNATLDPR

SEQ ID NO: 16 - protein, 19 aa, Artificial Sequence
  Peptide
RTRARRPESKATNATLDPR

SEQ ID NO: 17 - protein, 20 aa, Artificial Sequence
  Peptide
ARTRARRPESKATNATLDPR